European Patent Application EP 4 190 805 A2, published June 7, 2023. Title: IN VITRO CELL CULTURE METHODS FOR BETA-THALASSEMIA USING ACTIVIN TYPE II RECEPTOR LIGAND TRAPS. Applicant: Celgene Corporation. The sequence listing filed with the application follows.

SEQUENCE LISTING (47 sequences)

SEQ ID NO: 1 - protein, 513 aa, Homo sapiens
  source 1..513: note = human ActRIIA precursor polypeptide
MGAAAKLAFAVFLISCSSGAILGRSETQECLFFNANWEKDRTNQTGVEPCYGDKDKRRHCFATWKNISGSIEIVKQGCWLDDINCYDRTDCVEKKDSPEVYFCCCEGNMCNEKFSYFPEMEVTQPTSNPVTPKPPYYNILLYSLVPLMLIAGIVICAFWVYRHHKMAYPPVLVPTQDPGPPPPSPLLGLKPLQLLEVKARGRFGCVWKAQLLNEYVAVKIFPIQDKQSWQNEYEVYSLPGMKHENILQFIGAEKRGTSVDVDLWLITAFHEKGSLSDFLKANVVSWNELCHIAETMARGLAYLHEDIPGLKDGHKPAISHRDIKSKNVLLKNNLTACIADFGLALKFEAGKSAGDTHGQVGTRRYMAPEVLEGAINFQRDAFLRIDMYAMGLVLWELASRCTAADGPVDEYMLPFEEEIGQHPSLEDMQEVVVHKKKRPVLRDYWQKHAGMAMLCETIEECWDHDAEARLSAGCVGERITQMQRLTNIITTEDIVTVVTMVTNVDFPPKESSL

SEQ ID NO: 2 - protein, 115 aa, Homo sapiens
  source 1..115: note = human ActRIIA soluble (extracellular), processed polypeptidesequence
ILGRSETQECLFFNANWEKDRTNQTGVEPCYGDKDKRRHCFATWKNISGSIEIVKQGCWLDDINCYDRTDCVEKKDSPEVYFCCCEGNMCNEKFSYFPEMEVTQPTSNPVTPKPP

SEQ ID NO: 3 - protein, 100 aa, synthetic construct
  source 1..100: note = human ActRIIA soluble (extracellular), processed polypeptidesequence with the C-terminal 15 amino acids deleted
ILGRSETQECLFFNANWEKDRTNQTGVEPCYGDKDKRRHCFATWKNISGSIEIVKQGCWLDDINCYDRTDCVEKKDSPEVYFCCCEGNMCNEKFSYFPEM

SEQ ID NO: 4 - DNA, 1542 bp, Homo sapiens
  source 1..1542: mol_type = other DNA; note = nucleic acid sequence of human ActRIIA precursor protein
atgggagctgctgcaaagttggcgtttgccgtctttcttatctcctgttcttcaggtgctatacttggtagatcagaaactcaggagtgtcttttctttaatgctaattgggaaaaagacagaaccaatcaaactggtgttgaaccgtgttatggtgacaaagataaacggcggcattgttttgctacctggaagaatatttctggttccattgaaatagtgaaacaaggttgttggctggatgatatcaactgctatgacaggactgattgtgtagaaaaaaaagacagccctgaagtatatttttgttgctgtgagggcaatatgtgtaatgaaaagttttcttattttccagagatggaagtcacacagcccacttcaaatccagttacacctaagccaccctattacaacatcctgctctattccttggtgccacttatgttaattgcggggattgtcatttgtgcattttgggtgtacaggcatcacaagatggcctaccctcctgtacttgttccaactcaagacccaggaccacccccaccttctccattactagggttgaaaccactgcagttattagaagtgaaagcaaggggaagatttggttgtgtctggaaagcccagttgcttaacgaatatgtggctgtcaaaatatttccaatacaggacaaacagtcatggcaaaatgaatacgaagtctacagtttgcctggaatgaagcatgagaacatattacagttcattggtgcagaaaaacgaggcaccagtgttgatgtggatctttggctgatcacagcatttcatgaaaagggttcactatcagactttcttaaggctaatgtggtctcttggaatgaactgtgtcatattgcagaaaccatggctagaggattggcatatttacatgaggatatacctggcctaaaagatggccacaaacctgccatatctcacagggacatcaaaagtaaaaatgtgctgttgaaaaacaacctgacagcttgcattgctgactttgggttggccttaaaatttgaggctggcaagtctgcaggcgatacccatggacaggttggtacccggaggtacatggctccagaggtattagagggtgctataaacttcgaaagggatgcatttttgaggatagatatgtatgccatgggattagtcctatgggaactggcttctcgctgtactgctgcagatggacctgtagatgaatacatgttgccatttgaggaggaaattggccagcatccatctcttgaagacatgcaggaagttgttgtgcataaaaaaaagaggcctgttttaagagattattggcagaaacatgctggaatggcaatgctctgtgaaaccattgaagaatgttgggatcacgacgcagaagccaggttatcagctggatgtgtaggtgaaagaattacccagatgcagagactaacaaatattattaccacagaggacattgtaacagtggtcacaatggtgacaaatgttgactttcctcccaaagaatctagtctatga

SEQ ID NO: 5 - DNA, 345 bp, Homo sapiens
  source 1..345: mol_type = other DNA; note = human ActRIIA soluble (extracellular) polypeptide
atacttggtagatcagaaactcaggagtgtcttttctttaatgctaattgggaaaaagacagaaccaatcaaactggtgttgaaccgtgttatggtgacaaagataaacggcggcattgttttgctacctggaagaatatttctggttccattgaaatagtgaaacaaggttgttggctggatgatatcaactgctatgacaggactgattgtgtagaaaaaaaagacagccctgaagtatatttttgttgctgtgagggcaatatgtgtaatgaaaagttttcttattttccagagatggaagtcacacagcccacttcaaatccagttacacctaagccaccc

SEQ ID NO: 6 - protein, 228 aa, synthetic construct
  VARIANT 44: note = Xaa = Asp or Ala
  VARIANT 102: note = Xaa = Lys or Ala
  VARIANT 215: note = Xaa = Asn or Ala
  source 1..228: note = fusion protein comprising a soluble extracellular domain of ActRIIA fused to an Fc domain
THTCPPCPAPELLGGPSVFLFPPKPKDTLMISRTPEVTCVVVDXVSHEDPEVKFNWYVDGVEVHNAKTKPREEQYNSTYRVVSVLTVLHQDWLNGKEYKCKXVSNKALPVPIEKTISKAKGQPREPQVYTLPPSREEMTKNQVSLTCLVKGFYPSDIAVEWESNGQPENNYKTTPPVLDSDGPFFLYSKLTVDKSRWQQGNVFSCSVMHEALHNXHYTQKSLSLSPGK

SEQ ID NO: 7 - protein, 344 aa, synthetic construct
  source 1..344: note = Extracellular domain of human ActRIIA fused to a humanFc domain
ILGRSETQECLFFNANWEKDRTNQTGVEPCYGDKDKRRHCFATWKNISGSIEIVKQGCWLDDINCYDRTDCVEKKDSPEVYFCCCEGNMCNEKFSYFPEMEVTQPTSNPVTPKPPTGGGTHTCPPCPAPELLGGPSVFLFPPKPKDTLMISRTPEVTCVVVDVSHEDPEVKFNWYVDGVEVHNAKTKPREEQYNSTYRVVSVLTVLHQDWLNGKEYKCKVSNKALPVPIEKTISKAKGQPREPQVYTLPPSREEMTKNQVSLTCLVKGFYPSDIAVEWESNGQPENNYKTTPPVLDSDGSFFLYSKLTVDKSRWQQGNVFSCSVMHEALHNHYTQKSLSLSPGK

SEQ ID NO: 8 - protein, 21 aa, synthetic construct
  source 1..21: note = Leader sequence of Honey bee mellitin (HBML)
MKFLVNVALVFMVVYISYIYA

SEQ ID NO: 9 - protein, 22 aa, synthetic construct
  source 1..22: note = Leader sequence of Tissue Plasminogen Activator (TPA)
MDAMKRGLCCVLLLCGAVFVSP

SEQ ID NO: 10 - protein, 20 aa, synthetic construct
  source 1..20: note = Native ActRIIA leader
MGAAAKLAFAVFLISCSSGA

SEQ ID NO: 11 - protein, 9 aa, synthetic construct
  source 1..9: note = ActRIIA-hFc and mActRIIA-Fc N-terminal sequence
ILGRSETQE

SEQ ID NO: 12 - protein, 329 aa, synthetic construct
  source 1..329: note = ActRIIA-Fc Protein with deletion of the C-terminal 15 aminoacids of the extracellular domain of ActRIIA
ILGRSETQECLFFNANWEKDRTNQTGVEPCYGDKDKRRHCFATWKNISGSIEIVKQGCWLDDINCYDRTDCVEKKDSPEVYFCCCEGNMCNEKFSYFPEMTGGGTHTCPPCPAPELLGGPSVFLFPPKPKDTLMISRTPEVTCVVVDVSHEDPEVKFNWYVDGVEVHNAKTKPREEQYNSTYRVVSVLTVLHQDWLNGKEYKCKVSNKALPVPIEKTISKAKGQPREPQVYTLPPSREEMTKNQVSLTCLVKGFYPSDIAVEWESNGQPENNYKTTPPVLDSDGSFFLYSKLTVDKSRWQQGNVFSCSVMHEALHNHYTQKSLSLSPGK

SEQ ID NO: 13 - protein, 369 aa, synthetic construct
  source 1..369: note = Unprocessed ActRIIA-hFc with TPA leader sequence
MDAMKRGLCCVLLLCGAVFVSPGAAILGRSETQECLFFNANWEKDRTNQTGVEPCYGDKDKRRHCFATWKNISGSIEIVKQGCWLDDINCYDRTDCVEKKDSPEVYFCCCEGNMCNEKFSYFPEMEVTQPTSNPVTPKPPTGGGTHTCPPCPAPELLGGPSVFLFPPKPKDTLMISRTPEVTCVVVDVSHEDPEVKFNWYVDGVEVHNAKTKPREEQYNSTYRVVSVLTVLHQDWLNGKEYKCKVSNKALPVPIEKTISKAKGQPREPQVYTLPPSREEMTKNQVSLTCLVKGFYPSDIAVEWESNGQPENNYKTTPPVLDSDGSFFLYSKLTVDKSRWQQGNVFSCSVMHEALHNHYTQKSLSLSPGK

SEQ ID NO: 14 - DNA, 1113 bp, synthetic construct
  source 1..1113: mol_type = other DNA; note = Nucleic acid sequence encoding Unprocessed ActRIIA-hFc with TPA leader sequence
atggatgcaatgaagagagggctctgctgtgtgctgctgctgtgtggagcagtcttcgtttcgcccggcgccgctatacttggtagatcagaaactcaggagtgtctttttttaatgctaattgggaaaaagacagaaccaatcaaactggtgttgaaccgtgttatggtgacaaagataaacggcggcattgttttgctacctggaagaatatttctggttccattgaatagtgaaacaaggttgttggctggatgatatcaactgctatgacaggactgattgtgtagaaaaaaaagacagccctgaagtatatttctgttgctgtgagggcaatatgtgtaatgaaaagttttcttattttccggagatggaagtcacacagcccacttcaaatccagttacacctaagccacccaccggtggtggaactcacacatgcccaccgtgcccagcacctgaactcctggggggaccgtcagtcttcctcttccccccaaaacccaaggacaccctcatgatctcccggacccctgaggtcacatgcgtggtggtggacgtgagccacgaagaccctgaggtcaagttcaactggtacgtggacggcgtggaggtgcataatgccaagacaaagccgcgggaggagcagtacaacagcacgtaccgtgtggtcagcgtcctcaccgtcctgcaccaggactggctgaatggcaaggagtacaagtgcaaggtctccaacaaagccctcccagtccccatcgagaaaaccatctccaaagccaaagggcagccccgagaaccacaggtgtacaccctgcccccatcccgggaggagatgaccaagaaccaggtcagcctgacctgcctggtcaaaggcttctatcccagcgacatcgccgtggagtgggagagcaatgggcagccggagaacaactacaagaccacgcctcccgtgctggactccgacggctccttcttcctctatagcaagctcaccgtggacaagagcaggtggcagcaggggaacgtcttctcatgctccgtgatgcatgaggctctgcacaaccactacacgcagaagagcctctccctgtctccggtaaatgagaattc

SEQ ID NO: 15 - protein, 106 aa, synthetic construct
  source 1..106: note = human ActRIIB soluble (extracellular processed polypeptide with the N-terminal 6 aa of the EC domain deleted and the C-terminal 4 aa of the EC domain deleted (aa 25-130 of SEQ ID NO:28) and with an L79D mutation
ETRECIYYNANWELERTNQSGLERCEGEQDKRLHCYASWRNSSGTIELVKKGCWDDDFNCYDRQECVATEENPQVYFCCCEGNFCNERFTHLPEAGGPEVTYEPPP

SEQ ID NO: 16 - protein, 512 aa, Homo sapiens
  source 1..512: note = human ActRIIB precursor protein sequence (A64)
MTAPWVALALLWGSLWPGSGRGEAETRECIYYNANWELERTNQSGLERCEGEQDKRLHCYASWANSSGTIELVKKGCWLDDFNCYDRQECVATEENPQVYFCCCEGNFCNERFTHLPEAGGPEVTYEPPPTAPTLLTVLAYSLLPIGGLSLIVLLAFWMYRHRKPPYGHVDIHEDPGPPPPSPLVGLKPLQLLEIKARGRFGCVWKAQLMNDFVAVKIFPLQDKQSWQSEREIFSTPGMKHENLLQFIAAEKRGSNLEVELWLITAFHDKGSLTDYLKGNIITWNELCHVAETMSRGLSYLHEDVPWCRGEGHKPSIAHRDFKSKNVLLKSDLTAVLADFGLAVRFEPGKPPGDTHGQVGTRRYMAPEVLEGAINFQRDAFLRIDMYAMGLVLWELVSRCKAADGPVDEYMLPFEEEIGQHPSLEELQEVVVHKKMRPTIKDHWLKHPGLAQLCVTIEECWDHDAEARLSAGCVEERVSLIRRSVNGTTSDCLVSLVTSVTNVDLPPKESSI

SEQ ID NO: 17 - protein, 116 aa, Homo sapiens
  source 1..116: note = human ActRIIB soluble (extracellular), processed polypeptide sequence (amino acids 19-134 of SEQ ID NO:16)
SGRGEAETRECIYYNANWELERTNQSGLERCEGEQDKRLHCYASWANSSGTIELVKKGCWLDDFNCYDRQECVATEENPQVYFCCCEGNFCNERFTHLPEAGGPEVTYEPPPTAPT

SEQ ID NO: 18 - protein, 101 aa, synthetic construct
  source 1..101: note = human ActRIIB soluble (extracellular) processed polypeptide with the C-terminal 15 aa deleted (aa 19-119 of SEQ ID NO:16)
SGRGEAETRECIYYNANWELERTNQSGLERCEGEQDKRLHCYASWANSSGTIELVKKGCWLDDFNCYDRQECVATEENPQVYFCCCEGNFCNERFTHLPEA

SEQ ID NO: 19 - DNA, 1539 bp, Homo sapiens
  source 1..1539: mol_type = other DNA; note = nucleic acid sequence encoding a human ActRIIB (A64) precursorprotein
atgacggcgccctgggtggccctcgccctcctctggggatcgctgtggcccggctctgggcgtggggaggctgagacacgggagtgcatctactacaacgccaactgggagctggagcgcaccaaccagagcggcctggagcgctgcgaaggcgagcaggacaagcggctgcactgctacgcctcctgggccaacagctctggcaccatcgagctcgtgaagaagggctgctggctagatgacttcaactgctacgataggcaggagtgtgtggccactgaggagaacccccaggtgtacttctgctgctgtgaaggcaacttctgcaacgagcgcttcactcatttgccagaggctgggggcccggaagtcacgtacgagccacccccgacagcccccaccctgctcacggtgctggcctactcactgctgcccatcgggggcctttccctcatcgtcctgctggccttttggatgtaccggcatcgcaagcccccctacggtcatgtggacatccatgaggaccctgggcctccaccaccatcccctctggtgggcctgaagccactgcagctgctggagatcaaggctcgggggcgctttggctgtgtctggaaggcccagctcatgaatgactttgtagctgtcaagatcttcccactccaggacaagcagtcgtggcagagtgaacgggagatcttcagcacacctggcatgaagcacgagaacctgctacagttcattgctgccgagaagcgaggctccaacctcgaagtagagctgtggctcatcacggccttccatgacaagggctccctcacggattacctcaaggggaacatcatcacatggaacgaactgtgtcatgtagcagagacgatgtcacgaggcctctcatacctgcatgaggatgtgccctggtgccgtggcgagggccacaagccgtctattgcccacagggactttaaaagtaagaatgtattgctgaagagcgacctcacagccgtgctggctgactttggcttggctgttcgatttgagccagggaaacctccaggggacacccacggacaggtaggcacgagacggtacatggctcctgaggtgctcgagggagccatcaacttccagagagatgccttcctgcgcattgacatgtatgccatggggttggtgctgtgggagcttgtgtctcgctgcaaggctgcagacggacccgtggatgagtacatgctgccctttgaggaagagattggccagcacccttcgttggaggagctgcaggaggtggtggtgcacaagaagatgaggcccaccattaaagatcactggttgaaacacccgggcctggcccagctttgtgtgaccatcgaggagtgctgggaccatgatgcagaggctcgcttgtccgcgggctgtgtggaggagcgggtgtccctgattcggaggtcggtcaacggcactacctcggactgtctcgtttccctggtgacctctgtcaccaatgtggacctgccccctaaagagtcaagcatctaa

SEQ ID NO: 20 - protein, 344 aa, synthetic construct
  source 1..344: note = fusion protein comprising a soluble extracellular domain of ActRIIB (A64; SEQ ID NO:17) fused to an Fc domain
SGRGEAETRECIYYNANWELERTNQSGLERCEGEQDKRLHCYASWANSSGTIELVKKGCWLDDFNCYDRQECVATEENPQVYFCCCEGNFCNERFTHLPEAGGPEVTYEPPPTAPTGGGTHTCPPCPAPELLGGPSVFLFPPKPKDTLMISRTPEVTCVVVDVSHEDPEVKFNWYVDGVEVHNAKTKPREEQYNSTYRVVSVLTVLHQDWLNGKEYKCKVSNKALPVPIEKTISKAKGQPREPQVYTLPPSREEMTKNQVSLTCLVKGFYPSDIAVEWESNGQPENNYKTTPPVLDSDGSFFLYSKLTVDKSRWQQGNVFSCSVMHEALHNHYTQKSLSLSPGK

SEQ ID NO: 21 - protein, 329 aa, synthetic construct
  source 1..329: note = fusion protein comprising a soluble extracellular domain of ActRIIB (A64) with the C-terminal 15 amino acids deleted (SEQ ID NO:18) fused to an Fc domain
SGRGEAETRECIYYNANWELERTNQSGLERCEGEQDKRLHCYASWANSSGTIELVKKGCWLDDFNCYDRQECVATEENPQVYFCCCEGNFCNERFTHLPEAGGGTHTCPPCPAPELLGGPSVFLFPPKPKDTLMISRTPEVTCVVVDVSHEDPEVKFNWYVDGVEVHNAKTKPREEQYNSTYRVVSVLTVLHQDWLNGKEYKCKVSNKALPVPIEKTISKAKGQPREPQVYTLPPSREEMTKNQVSLTCLVKGFYPSDIAVEWESNGQPENNYKTTPPVLDSDGSFFLYSKLTVDKSRWQQGNVFSCSVMHEALHNHYTQKSLSLSPGK

SEQ ID NO: 22 - protein, 105 aa, synthetic construct
  source 1..105: note = human ActRIIB soluble (extracellular) processed polypeptide with the N-terminal 6 aa of the EC domain deleted and the C-terminal 5 aa of the EC domain deleted (aa 25-129 of SEQ ID NO:28) and with an L79D mutation
ETRECIYYNANWELERTNQSGLERCEGEQDKRLHCYASWRNSSGTIELVKKGCWDDDFNCYDRQECVATEENPQVYFCCCEGNFCNERFTHLPEAGGPEVTYEPP

SEQ ID NO: 23 - protein, 107 aa, synthetic construct
  source 1..107: note = human ActRIIB soluble (extracellular) processed polypeptide with the N-terminal 6 aa of the EC domain deleted and the C-terminal 3 aa of the EC domain deleted (aa 25-131 of SEQ ID NO:28) and with an L79D mutation
ETRECIYYNANWELERTNQSGLERCEGEQDKRLHCYASWRNSSGTIELVKKGCWDDDFNCYDRQECVATEENPQVYFCCCEGNFCNERFTHLPEAGGPEVTYEPPPT

SEQ ID NO: 24 - protein, 360 aa, synthetic construct
  source 1..360: note = Unprocessed ActRIIB-Fc fusion protein with the N-terminal 6 aa of the EC domain deleted and the C-terminal 3 aa of the EC domain deleted (aa 25-131 of SEQ ID NO:28) and with an L79D mutation and with TPA leader sequence
MDAMKRGLCCVLLLCGAVFVSPGAAETRECIYYNANWELERTNQSGLERCEGEQDKRLHCYASWRNSSGTIELVKKGCWDDDFNCYDRQECVATEENPQVYFCCCEGNFCNERFTHLPEAGGPEVTYEPPPTGGGTHTCPPCPAPELLGGPSVFLFPPKPKDTLMISRTPEVTCVVVDVSHEDPEVKFNWYVDGVEVHNAKTKPREEQYNSTYRVVSVLTVLHQDWLNGKEYKCKVSNKALPAPIEKTISKAKGQPREPQVYTLPPSREEMTKNQVSLTCLVKGFYPSDIAVEWESNGQPENNYKTTPPVLDSDGSFFLYSKLTVDKSRWQQGNVFSCSVMHEALHNHYTQKSLSLSPGK

SEQ ID NO: 25 - protein, 335 aa, synthetic construct
  source 1..335: note = Processed ActRIIB-Fc fusion protein with the N-terminal 6 aa of the EC domain deleted and the C-terminal 3 aa of the EC domain deleted (aa 25-131 of SEQ ID NO:28) and with an L79D mutation
ETRECIYYNANWELERTNQSGLERCEGEQDKRLHCYASWRNSSGTIELVKKGCWDDDFNCYDRQECVATEENPQVYFCCCEGNFCNERFTHLPEAGGPEVTYEPPPTGGGTHTCPPCPAPELLGGPSVFLFPPKPKDTLMISRTPEVTCVVVDVSHEDPEVKFNWYVDGVEVHNAKTKPREEQYNSTYRVVSVLTVLHQDWLNGKEYKCKVSNKALPAPIEKTISKAKGQPREPQVYTLPPSREEMTKNQVSLTCLVKGFYPSDIAVEWESNGQPENNYKTTPPVLDSDGSFFLYSKLTVDKSRWQQGNVFSCSVMHEALHNHYTQKSLSLSPGK

SEQ ID NO: 26 - protein, 115 aa, Homo sapiens
  source 1..115: note = human ActRIIB soluble (extracellular), processed polypeptide sequence (amino acids 20-134 of SEQ ID NO:16)
GRGEAETRECIYYNANWELERTNQSGLERCEGEQDKRLHCYASWANSSGTIELVKKGCWLDDFNCYDRQECVATEENPQVYFCCCEGNFCNERFTHLPEAGGPEVTYEPPPTAPT

SEQ ID NO: 27 - protein, 100 aa, synthetic construct
  source 1..100: note = human ActRIIB soluble (extracellular), processed polypeptide sequence with the C-terminal 15 aa deleted (aa 20-119 of SEQ ID NO:16)
GRGEAETRECIYYNANWELERTNQSGLERCEGEQDKRLHCYASWANSSGTIELVKKGCWLDDFNCYDRQECVATEENPQVYFCCCEGNFCNERFTHLPEA

SEQ ID NO: 28 - protein, 512 aa, Homo sapiens
  source 1..512: note = human ActRIIB precursor protein sequence (R64)
MTAPWVALALLWGSLWPGSGRGEAETRECIYYNANWELERTNQSGLERCEGEQDKRLHCYASWRNSSGTIELVKKGCWLDDFNCYDRQECVATEENPQVYFCCCEGNFCNERFTHLPEAGGPEVTYEPPPTAPTLLTVLAYSLLPIGGLSLIVLLAFWMYRHRKPPYGHVDIHEDPGPPPPSPLVGLKPLQLLEIKARGRFGCVWKAQLMNDFVAVKIFPLQDKQSWQSEREIFSTPGMKHENLLQFIAAEKRGSNLEVELWLITAFHDKGSLTDYLKGNIITWNELCHVAETMSRGLSYLHEDVPWCRGEGHKPSIAHRDFKSKNVLLKSDLTAVLADFGLAVRFEPGKPPGDTHGQVGTRRYMAPEVLEGAINFQRDAFLRIDMYAMGLVLWELVSRCKAADGPVDEYMLPFEEEIGQHPSLEELQEVVVHKKMRPTIKDHWLKHPGLAQLCVTIEECWDHDAEARLSAGCVEERVSLIRRSVNGTTSDCLVSLVTSVTNVDLPPKESSI

SEQ ID NO: 29 - protein, 116 aa, synthetic construct
  source 1..116: note = human ActRIIB soluble (extracellular), processed polypeptide sequence (amino acids 19-134 of SEQ ID NO:28)
SGRGEAETRECIYYNANWELERTNQSGLERCEGEQDKRLHCYASWRNSSGTIELVKKGCWLDDFNCYDRQECVATEENPQVYFCCCEGNFCNERFTHLPEAGGPEVTYEPPPTAPT

SEQ ID NO: 30 - protein, 101 aa, synthetic construct
  source 1..101: note = human ActRIIB soluble (extracellular), processed polypeptide sequence with the C-terminal 15 aa deleted (aa 19-119 of SEQ ID NO:28)
SGRGEAETRECIYYNANWELERTNQSGLERCEGEQDKRLHCYASWRNSSGTIELVKKGCWLDDFNCYDRQECVATEENPQVYFCCCEGNFCNERFTHLPEA

SEQ ID NO: 31 - protein, 115 aa, synthetic construct
  source 1..115: note = human ActRIIB soluble (extracellular), processed polypeptide sequence (amino acids 20-134 of SEQ ID NO:28)
GRGEAETRECIYYNANWELERTNQSGLERCEGEQDKRLHCYASWRNSSGTIELVKKGCWLDDFNCYDRQECVATEENPQVYFCCCEGNFCNERFTHLPEAGGPEVTYEPPPTAPT

SEQ ID NO: 32 - protein, 100 aa, synthetic construct
  source 1..100: note = human ActRIIB soluble (extracellular), processed polypeptide sequence with the C-terminal 15 aa deleted (aa 20-119 of SEQ ID NO:28)
GRGEAETRECIYYNANWELERTNQSGLERCEGEQDKRLHCYASWRNSSGTIELVKKGCWLDDFNCYDRQECVATEENPQVYFCCCEGNFCNERFTHLPEA

SEQ ID NO: 33 - protein, 107 aa, synthetic construct
  source 1..107: note = human ActRIIB soluble (extracellular) processed polypeptide with the N-terminal 6 aa of the EC domain deleted and the C-terminal 3 aa of the EC domain deleted (aa 25-131 of SEQ ID NO:16) and with an L79D mutation
ETRECIYYNANWELERTNQSGLERCEGEQDKRLHCYASWANSSGTIELVKKGCWDDDFNCYDRQECVATEENPQVYFCCCEGNFCNERFTHLPEAGGPEVTYEPPPT

SEQ ID NO: 34 - protein, 360 aa, synthetic construct
  source 1..360: note = Unprocessed ActRIIB-Fc fusion protein with the N-terminal 6 aa of the EC domain deleted and the C-terminal 3 aa of the EC domain deleted (aa 25-131 of SEQ ID NO:16) and with an L79D mutation and with TPA leader sequence
MDAMKRGLCCVLLLCGAVFVSPGAAETRECIYYNANWELERTNQSGLERCEGEQDKRLHCYASWANSSGTIELVKKGCWDDDFNCYDRQECVATEENPQVYFCCCEGNFCNERFTHLPEAGGPEVTYEPPPTGGGTHTCPPCPAPELLGGPSVFLFPPKPKDTLMISRTPEVTCVVVDVSHEDPEVKFNWYVDGVEVHNAKTKPREEQYNSTYRVVSVLTVLHQDWLNGKEYKCKVSNKALPAPIEKTISKAKGQPREPQVYTLPPSREEMTKNQVSLTCLVKGFYPSDIAVEWESNGQPENNYKTTPPVLDSDGSFFLYSKLTVDKSRWQQGNVFSCSVMHEALHNHYTQKSLSLSPGK

SEQ ID NO: 35 - protein, 335 aa, synthetic construct
  source 1..335: note = Processed ActRIIB-Fc fusion protein with the N-terminal 6 aa of the EC domain deleted and the C-terminal 3 aa of the EC domain deleted (aa 25-131 of SEQ ID NO:16) and with an L79D mutation
ETRECIYYNANWELERTNQSGLERCEGEQDKRLHCYASWANSSGTIELVKKGCWDDDFNCYDRQECVATEENPQVYFCCCEGNFCNERFTHLPEAGGPEVTYEPPPTGGGTHTCPPCPAPELLGGPSVFLFPPKPKDTLMISRTPEVTCVVVDVSHEDPEVKFNWYVDGVEVHNAKTKPREEQYNSTYRVVSVLTVLHQDWLNGKEYKCKVSNKALPAPIEKTISKAKGQPREPQVYTLPPSREEMTKNQVSLTCLVKGFYPSDIAVEWESNGQPENNYKTTPPVLDSDGSFFLYSKLTVDKSRWQQGNVFSCSVMHEALHNHYTQKSLSLSPGK

SEQ ID NO: 36 - protein, 115 aa, synthetic construct
  source 1..115: note = human ActRIIB soluble (extracellular), processed polypeptide sequence (amino acids 20-134 of SEQ ID NO:28) with L79D mutation
GRGEAETRECIYYNANWELERTNQSGLERCEGEQDKRLHCYASWRNSSGTIELVKKGCWDDDFNCYDRQECVATEENPQVYFCCCEGNFCNERFTHLPEAGGPEVTYEPPPTAPT

SEQ ID NO: 37 - protein, 115 aa, synthetic construct
  source 1..115: note = human ActRIIB soluble (extracellular), processed polypeptide sequence (amino acids 20-134 of SEQ ID NO:16) with L79D mutation
GRGEAETRECIYYNANWELERTNQSGLERCEGEQDKRLHCYASWANSSGTIELVKKGCWDDDFNCYDRQECVATEENPQVYFCCCEGNFCNERFTHLPEAGGPEVTYEPPPTAPT

SEQ ID NO: 38 - protein, 343 aa, synthetic construct
  source 1..343: note = human ActRIIB soluble (extracellular), processed polypeptide sequence (aa 20-134 of SEQ ID NO:28) with L79D mutation fused to an Fc domain with a GGG linker
GRGEAETRECIYYNANWELERTNQSGLERCEGEQDKRLHCYASWRNSSGTIELVKKGCWDDDFNCYDRQECVATEENPQVYFCCCEGNFCNERFTHLPEAGGPEVTYEPPPTAPTGGGTHTCPPCPAPELLGGPSVFLFPPKPKDTLMISRTPEVTCVVVDVSHEDPEVKFNWYVDGVEVHNAKTKPREEQYNSTYRVVSVLTVLHQDWLNGKEYKCKVSNKALPAPIEKTISKAKGQPREPQVYTLPPSREEMTKNQVSLTCLVKGFYPSDIAVEWESNGQPENNYKTTPPVLDSDGSFFLYSKLTVDKSRWQQGNVFSCSVMHEALHNHYTQKSLSLSPGK

SEQ ID NO: 39 - protein, 343 aa, synthetic construct
  source 1..343: note = human ActRIIB soluble (extracellular), processed polypeptide sequence (aa 20-134 of SEQ ID NO:16) with L79D mutation fused to an Fc domain
GRGEAETRECIYYNANWELERTNQSGLERCEGEQDKRLHCYASWANSSGTIELVKKGCWDDDFNCYDRQECVATEENPQVYFCCCEGNFCNERFTHLPEAGGPEVTYEPPPTAPTGGGTHTCPPCPAPELLGGPSVFLFPPKPKDTLMISRTPEVTCVVVDVSHEDPEVKFNWYVDGVEVHNAKTKPREEQYNSTYRVVSVLTVLHQDWLNGKEYKCKVSNKALPAPIEKTISKAKGQPREPQVYTLPPSREEMTKNQVSLTCLVKGFYPSDIAVEWESNGQPENNYKTTPPVLDSDGSFFLYSKLTVDKSRWQQGNVFSCSVMHEALHNHYTQKSLSLSPGK

SEQ ID NO: 40 - protein, 368 aa, synthetic construct
  source 1..368: note = human ActRIIB soluble (extracellular), processed polypeptide sequence (aa 20-134 of SEQ ID NO:28) with L79D mutation fused to an Fc domain and with TPA leader sequence
MDAMKRGLCCVLLLCGAVFVSPGASGRGEAETRECIYYNANWELERTNQSGLERCEGEQDKRLHCYASWRNSSGTIELVKKGCWDDDFNCYDRQECVATEENPQVYFCCCEGNFCNERFTHLPEAGGPEVTYEPPPTAPTGGGTHTCPPCPAPELLGGPSVFLFPPKPKDTLMISRTPEVTCVVVDVSHEDPEVKFNWYVDGVEVHNAKTKPREEQYNSTYRVVSVLTVLHQDWLNGKEYKCKVSNKALPAPIEKTISKAKGQPREPQVYTLPPSREEMTKNQVSLTCLVKGFYPSDIAVEWESNGQPENNYKTTPPVLDSDGSFFLYSKLTVDKSRWQQGNVFSCSVMHEALHNHYTQKSLSLSPGK

SEQ ID NO: 41 - protein, 368 aa, synthetic construct
  source 1..368: note = human ActRIIB soluble (extracellular), processed polypeptide sequence (aa 20-134 of SEQ ID NO:16) with L79D mutation fused to an Fc domain and with TPA leader sequence
MDAMKRGLCCVLLLCGAVFVSPGASGRGEAETRECIYYNANWELERTNQSGLERCEGEQDKRLHCYASWANSSGTIELVKKGCWDDDFNCYDRQECVATEENPQVYFCCCEGNFCNERFTHLPEAGGPEVTYEPPPTAPTGGGTHTCPPCPAPELLGGPSVFLFPPKPKDTLMISRTPEVTCVVVDVSHEDPEVKFNWYVDGVEVHNAKTKPREEQYNSTYRVVSVLTVLHQDWLNGKEYKCKVSNKALPAPIEKTISKAKGQPREPQVYTLPPSREEMTKNQVSLTCLVKGFYPSDIAVEWESNGQPENNYKTTPPVLDSDGSFFLYSKLTVDKSRWQQGNVFSCSVMHEALHNHYTQKSLSLSPGK

SEQ ID NO: 42 - protein, 141 aa, synthetic construct
  source 1..141: note = human ActRIIB soluble (extracellular), processed polypeptide sequence having a variant C-terminal sequence (disclosed in WO2007/053775)
GRGEAETRECIYYNANWELERTNQSGLERCEGEQDKRLHCYASWRNSSGTIELVKKGCWLDDFNCYDRQECVATEENPQVYFCCCEGNFCNERFTHLPEAGGPEGPWASTTIPSGGPEATAAAGDQGSGALWLCLEGPAHE

SEQ ID NO: 43 - protein, 141 aa, synthetic construct
  source 1..141: note = human ActRIIB soluble (extracellular), processed polypeptide sequence having a variant C-terminal sequence (disclosed in WO2007/053775) having an L79D mutation
GRGEAETRECIYYNANWELERTNQSGLERCEGEQDKRLHCYASWRNSSGTIELVKKGCWDDDFNCYDRQECVATEENPQVYFCCCEGNFCNERFTHLPEAGGPEGPWASTTIPSGGPEATAAAGDQGSGALWLCLEGPAHE

SEQ ID NO: 44 - protein, 370 aa, synthetic construct
  source 1..370: note = human ActRIIB soluble (extracellular), processed polypeptide sequence having a variant C-terminal sequence (disclosed in WO2007/053775) having an L79D mutation fused to an Fc domain witha TGGG linker
GRGEAETRECIYYNANWELERTNQSGLERCEGEQDKRLHCYASWRNSSGTIELVKKGCWDDDFNCYDRQECVATEENPQVYFCCCEGNFCNERFTHLPEAGGPEGPWASTTIPSGGPEATAAAGDQGSGALWLCLEGPAHETGGGTHTCPPCPAPELLGGPSVFLFPPKPKDTLMISRTPEVTCVVVDVSHEDPEVKFNWYVDGVEVHNAKTKPREEQYNSTYRVVSVLTVLHQDWLNGKEYKCKVSNKALPAPIEKTISKAKGQPREPQVYTLPPSREEMTKNQVSLTCLVKGFYPSDIAVEWESNGQPENNYKTTPPVLDSDGSFFLYSKLTVDKSRWQQGNVFSCSVMHEALHNHYTQKSLSLSPGK

SEQ ID NO: 45 - DNA, 1083 bp, synthetic construct
  source 1..1083: mol_type = other DNA; note = Nucleic Acid Sequence Encoding SEQ ID NO:24
atggatgcaatgaagagagggctctgctgtgtgctgctgctgtgtggagcagtcttcgtttcgcccggcgccgccgaaacccgcgaatgtatttattacaatgctaattgggaactcgaacggacgaaccaatccgggctcgaacggtgtgagggggaacaggataaacgcctccattgctatgcgtcgtggaggaactcctccgggacgattgaactggtcaagaaagggtgctgggacgacgatttcaattgttatgaccgccaggaatgtgtcgcgaccgaagagaatccgcaggtctatttctgttgttgcgaggggaatttctgtaatgaacggtttacccacctccccgaagccggcgggcccgaggtgacctatgaacccccgcccaccggtggtggaactcacacatgcccaccgtgcccagcacctgaactcctggggggaccgtcagtcttcctcttccccccaaaacccaaggacaccctcatgatctcccggacccctgaggtcacatgcgtggtggtggacgtgagccacgaagaccctgaggtcaagttcaactggtacgtggacggcgtggaggtgcataatgccaagacaaagccgcgggaggagcagtacaacagcacgtaccgtgtggtcagcgtcctcaccgtcctgcaccaggactggctgaatggcaaggagtacaagtgcaaggtctccaacaaagccctcccagcccccatcgagaaaaccatctccaaagccaaagggcagccccgagaaccacaggtgtacaccctgcccccatcccgggaggagatgaccaagaaccaggtcagcctgacctgcctggtcaaaggcttctatcccagcgacatcgccgtggagtgggagagcaatgggcagccggagaacaactacaagaccacgcctcccgtgctggactccgacggctccttcttcctctatagcaagctcaccgtggacaagagcaggtggcagcaggggaacgtcttctcatgctccgtgatgcatgaggctctgcacaaccactacacgcagaagagcctctccctgtccccgggtaaatga

SEQ ID NO: 46 - protein, 344 aa, synthetic construct
  source 1..344: note = fusion protein comprising a soluble extracellular domain of ActRIIB (R64; SEQ ID NO:29) fused to an Fc domain
SGRGEAETRECIYYNANWELERTNQSGLERCEGEQDKRLHCYASWRNSSGTIELVKKGCWLDDFNCYDRQECVATEENPQVYFCCCEGNFCNERFTHLPEAGGPEVTYEPPPTAPTGGGTHTCPPCPAPELLGGPSVFLFPPKPKDTLMISRTPEVTCVVVDVSHEDPEVKFNWYVDGVEVHNAKTKPREEQYNSTYRVVSVLTVLHQDWLNGKEYKCKVSNKALPVPIEKTISKAKGQPREPQVYTLPPSREEMTKNQVSLTCLVKGFYPSDIAVEWESNGQPENNYKTTPPVLDSDGSFFLYSKLTVDKSRWQQGNVFSCSVMHEALHNHYTQKSLSLSPGK

SEQ ID NO: 47 - protein, 329 aa, synthetic construct
  source 1..329: note = fusion protein comprising a soluble extracellular domain of ActRIIB (R64) with the C-terminal 15 aa deleted (SEQ ID NO:30) fused to an Fc domain
SGRGEAETRECIYYNANWELERTNQSGLERCEGEQDKRLHCYASWRNSSGTIELVKKGCWLDDFNCYDRQECVATEENPQVYFCCCEGNFCNERFTHLPEAGGGTHTCPPCPAPELLGGPSVFLFPPKPKDTLMISRTPEVTCVVVDVSHEDPEVKFNWYVDGVEVHNAKTKPREEQYNSTYRVVSVLTVLHQDWLNGKEYKCKVSNKALPVPIEKTISKAKGQPREPQVYTLPPSREEMTKNQVSLTCLVKGFYPSDIAVEWESNGQPENNYKTTPPVLDSDGSFFLYSKLTVDKSRWQQGNVFSCSVMHEALHNHYTQKSLSLSPGK